European Patent Specification EP 3 294 897 B1, published September 4, 2024. Title: A METHOD FOR PRODUCING RESVERATROL. Applicant: Evolva SA. The sequence listing filed with the application follows.

SEQUENCE LISTING (26 sequences)

SEQ ID NO: 1 - protein, 370 aa, Saccharomyces cerevisiae
MSESPMFAANGMPKVNQGAEEDVRILGYDPLASPALLQVQIPATPTSLETAKRGRREAIDIITGKDDRVLVIVGPCSIHDLEAAQEYALRLKKLSDELKGDLSIIMRAYLEKPRTTVGWKGLINDPDVNNTFNINKGLQSARQLFVNLTNIGLPIGSEMLDTISPQYLADLVSFGAIGARTTESQLHRELASGLSFPVGFKNGTDGTLNVAVDACQAAAHSHHFMGVTKHGVAAITTTKGNEHCFVILRGGKKGTNYDAKSVAEAKAQLPAGSNGLMIDYSHGNSNKDFRNQPKVNDVVCEQIANGENAITGVMIESNINEGNQGIPAEGKAGLKYGVSITDACIGWETTEDVLRKLAAAVRQRREVNKK

SEQ ID NO: 2 - protein, 370 aa, Saccharomyces cerevisiae
MSESPMFAANGMPKVNQGAEEDVRILGYDPLASPALLQVQIPATPTSLETAKRGRREAIDIITGKDDRVLVIVGPCSIHDLEAAQEYALRLKKLSDELKGDLSIIMRAYLEKPRTTVGWKGLINDPDVNNTFNINKGLQSARQLFVNLTNIGLPIGSEMLDTISPQYLADLVSFGAIGARTTESQLHRELASGLSFPVGFKNGTDGTLNVAVDACQAAAHSHHFMGVTLHGVAAITTTKGNEHCFVILRGGKKGTNYDAKSVAEAKAQLPAGSNGLMIDYSHGNSNKDFRNQPKVNDVVCEQIANGENAITGVMIESNINEGNQGIPAEGKAGLKYGVSITDACIGWETTEDVLRKLAAAVRQRREVNKK

SEQ ID NO: 3 - protein, 370 aa, Saccharomyces cerevisiae
MFIKNDHAGDRKRLEDWRIKGYDPLTPPDLLQHEFPISAKGEENIIKARDSVCDILNGKDDRLVIVIGPCSLHDPKAAYDYADRLAKISEKLSKDLLIIMRAYLEKPRTTVGWKGLINDPDMNNSFQINKGLRISREMFIKLVEKLPIAGEMLDTISPQFLSDCFSLGAIGARTTESQLHRELASGLSFPIGFKNGTDGGLQVAIDAMRAAAHEHYFLSVTKPGVTAIVGTEGNKDTFLILRGGKNGTNFDKESVQNTKKQLEKAGLTDDSQKRIMIDCSHGNSNKDFKNQPKVAKCIYDQLTEGENSLCGVMIESNINEGRQDIPKEGGREGLKYGCSVTDACIGWESTEQVLELLAEGVRNRRKALKK

SEQ ID NO: 4 - protein, 256 aa, Saccharomyces cerevisiae
MDFTKPETVLNLQNIRDELVRMEDSIIFKFIERSHFATCPSVYEANHPGLEIPNFKGSFLDWALSNLEIAHSRIRRFESPDETPFFPDKIQKSFLPSINYPQILAPYAPEVNYNDKIKKVYIEKIIPLISKRDGDDKNNFGSVATRDIECLQSLSRRIHFGKFVAEAKFQSDIPLYTKLIKSKDVEGIMKNITNSAVEEKILERLTKKAEVYGVDPTNESGERRITPEYLVKIYKEIVIPITKEVEVEYLLRRLEE

SEQ ID NO: 5 - protein, 256 aa, Saccharomyces cerevisiae
MDFTKPETVLNLQNIRDELVRMEDSIIFKFIERSHFATCPSVYEANHPGLEIPNFKGSFLDWALSNLEIAHSRIRRFESPDETPFFPDKIQKSFLPSINYPQILAPYAPEVNYNDKIKKVYIEKIIPLISKRDGDDKNNFGSVATRDIECLQSLSRRIHFGKFVAEAKFQSDIPLYTKLIKSKDVEGIMKNITNSAVEEKILERLTKKAEVYGVDPTNESGERRIIPEYLVKIYKEIVIPITKEVEVEYLLRRLEE

SEQ ID NO: 6 - protein, 2233 aa, Saccharomyces cerevisiae
MSEESLFESSPQKMEYEITNYSERHTELPGHFIGLNTVDKLEESPLRDFVKSHGGHTVISKILIANNGIAAVKEIRSVRKWAYETFGDDRTVQFVAMATPEDLEANAEYIRMADQYIEVPGGTNNNNYANVDLIVDIAERADVDAVWAGWGHASENPLLPEKLSQSKRKVIFIGPPGNAMRSLGDKISSTIVAQSAKVPCIPWSGTGVDTVHVDEKTGLVSVDDDIYQKGCCTSPEDGLQKAKRIGFPVMIKASEGGGGKGIRQVEREEDFIALYHQAANEIPGSPIFIMKLAGRARHLEVQLLADQYGTNISLFGRDCSVQRRHQKIIEEAPVTIAKAETFHEMEKAAVRLGKLVGYVSAGTVEYLYSHDDGKFYFLELNPRLQVEHPTTEMVSGVNLPAAQLQIAMGIPMHRISDIRTLYGMNPHSASEIDFEFKTQDATKKQRRPIPKGHCTACRITSEDPNDGFKPSGGTLHELNFRSSSNVWGYFSVGNNGNIHSFSDSQFGHIFAFGENRQASRKHMVVALKELSIRGDFRTTVEYLIKLLETEDFEDNTITTGWLDDLITHKMTAEKPDPTLAVICGAATKAFLASEEARHKYIESLQKGQVLSKDLLQTMFPVDFIHEGKRYKFTVAKSGNDRYTLFINGSKCDIILRQLSDGGLLIAIGGKSHTIYWKEEVAATRLSVDSMTTLLEVENDPTQLRTPSPGKLVKFLVENGEHIIKGQPYAEIEVMKMQMPLVSQENGIVQLLKQPGSTIVAGDIMAIMTLDDPSKVKHALPFEGMLPDFGSPVIEGTKPAYKFKSLVSTLENILKGYDNQVIMNASLQQLIEVLRNPKLPYSEWKLHISALHSRLPAKLDEQMEELVARSLRRGAVFPARQLSKLIDMAVKNPEYNPDKLLGAVVEPLADIAHKYSNGLEAHEHSIFVHFLEEYYEVEKLFNGPNVREENIILKLRDENPKDLDKVALTVLSHSKVSAKNNLILAILKHYQPLCKLSSKVSAIFSTPLQHIVELESKATAKVALQAREILIQGALPSVKERTEQIEHILKSSVVKVAYGSSNPKRSEPDLNILKDLIDSNYVVFDVLLQFLTHQDPVVTAAAAQVYIRRAYRAYTIGDIRVHEGVTVPIVEWKFQLPSAAFSTFPTVKSKMGMNRAVSVSDLSYVANSQSSPLREGILMAVDHLDDVDEILSQSLEVIPRHQSSSNGPAPDRSGSSASLSNVANVCVASTEGFESEEEILVRLREILDLNKQELINASIRRITFMFGFKDGSYPKYYTFNGPNYNENETIRHIEPALAFQLELGRLSNFNIKPIFTDNRNIHVYEAVSKTSPLDKRFFTRGIIRTGHIRDDISIQEYLTSEANRLMSDILDNLEVTDTSNSDLNHIFINFIAVFDISPEDVEAAFGGFLERFGKRLLRLRVSSAEIRIIIKDPQTGAPVPLRALINNVSGYVIKTEMYTEVKNAKGEWVFKSLGKPGSMHLRPIATPYPVKEWLQPKRYKAHLMGTTYVYDFPELFRQASSSQWKNFSADVKLTDDFFISNELIEDENGELTEVEREPGANAIGMVAFKITVKTPEYPRGRQFVVVANDITFKIGSFGPQEDEFFNKVTEYARKRGIPRIYLAANSGARIGMAEEIVPLFQVAWNDAANPDKGFQYLYLTSEGMETLKKFDKENSVLTERTVINGEERFVIKTIIGSEDGLGVECLRGSGLIAGATSRAYHDIFTITLVTCRSVGIGAYLVRLGQRAIQVEGQPIILTGAPAINKMLGREVYTSNLQLGGTQIMYNNGVSHLTAVDDLAGVEKIVEWMSYVPAKRNMPVPILETKDTWDRPVDFTPTNDETYDVRWMIEGRETESGFEYGLFDKGSFFETLSGWAKGVVVGRARLGGIPLGVIGVETRTVENLIPADPANPNSAETLIQEPGQVWHPNSAFKTAQAINDFNNGEQLPMMILANWRGFSGGQRDMFNEVLKYGSFIVDALVDYKQPIIIYIPPTGELRGGSWVVVDPTINADQMEMYADVNARAGVLEPQGMVGIKFRREKLLDTMNRLDDKYRELRSQLSNKSLAPEVHQQISKQLADRERELLPIYGQISLQFADLHDRSSRMVAKGVISKELEWTEARRFFFWRLRRRLNEEYLIKRLSHQVGEASRLEKIARIRSWYPASVDHEDDRQVATWIEENYKTLDDKLKGLKLESFAQDLAKKIRSDHDNAIDGLSEVIKMLSTDDKEKLLKTLK

SEQ ID NO: 7 - protein, 2233 aa, Artificial Sequence
  S. cerevisiae ACC1 S659A
MSEESLFESSPQKMEYEITNYSERHTELPGHFIGLNTVDKLEESPLRDFVKSHGGHTVISKILIANNGIAAVKEIRSVRKWAYETFGDDRTVQFVAMATPEDLEANAEYIRMADQYIEVPGGTNNNNYANVDLIVDIAERADVDAVWAGWGHASENPLLPEKLSQSKRKVIFIGPPGNAMRSLGDKISSTIVAQSAKVPCIPWSGTGVDTVHVDEKTGLVSVDDDIYQKGCCTSPEDGLQKAKRIGFPVMIKASEGGGGKGIRQVEREEDFIALYHQAANEIPGSPIFIMKLAGRARHLEVQLLADQYGTNISLFGRDCSVQRRHQKIIEEAPVTIAKAETFHEMEKAAVRLGKLVGYVSAGTVEYLYSHDDGKFYFLELNPRLQVEHPTTEMVSGVNLPAAQLQIAMGIPMHRISDIRTLYGMNPHSASEIDFEFKTQDATKKQRRPIPKGHCTACRITSEDPNDGFKPSGGTLHELNFRSSSNVWGYFSVGNNGNIHSFSDSQFGHIFAFGENRQASRKHMVVALKELSIRGDFRTTVEYLIKLLETEDFEDNTITTGWLDDLITHKMTAEKPDPTLAVICGAATKAFLASEEARHKYIESLQKGQVLSKDLLQTMFPVDFIHEGKRYKFTVAKSGNDRYTLFINGSKCDIILRQLADGGLLIAIGGKSHTIYWKEEVAATRLSVDSMTTLLEVENDPTQLRTPSPGKLVKFLVENGEHIIKGQPYAEIEVMKMQMPLVSQENGIVQLLKQPGSTIVAGDIMAIMTLDDPSKVKHALPFEGMLPDFGSPVIEGTKPAYKFKSLVSTLENILKGYDNQVIMNASLQQLIEVLRNPKLPYSEWKLHISALHSRLPAKLDEQMEELVARSLRRGAVFPARQLSKLIDMAVKNPEYNPDKLLGAVVEPLADIAHKYSNGLEAHEHSIFVHFLEEYYEVEKLFNGPNVREENIILKLRDENPKDLDKVALTVLSHSKVSAKNNLILAILKHYQPLCKLSSKVSAIFSTPLQHIVELESKATAKVALQAREILIQGALPSVKERTEQIEHILKSSVVKVAYGSSNPKRSEPDLNILKDLIDSNYVVFDVLLQFLTHQDPVVTAAAAQVYIRRAYRAYTIGDIRVHEGVTVPIVEWKFQLPSAAFSTFPTVKSKMGMNRAVSVSDLSYVANSQSSPLREGILMAVDHLDDVDEILSQSLEVIPRHQSSSNGPAPDRSGSSASLSNVANVCVASTEGFESEEEILVRLREILDLNKQELINASIRRITFMFGFKDGSYPKYYTFNGPNYNENETIRHIEPALAFQLELGRLSNFNIKPIFTDNRNIHVYEAVSKTSPLDKRFFTRGIIRTGHIRDDISIQEYLTSEANRLMSDILDNLEVTDTSNSDLNHIFINFIAVFDISPEDVEAAFGGFLERFGKRLLRLRVSSAEIRIIIKDPQTGAPVPLRALINNVSGYVIKTEMYTEVKNAKGEWVFKSLGKPGSMHLRPIATPYPVKEWLQPKRYKAHLMGTTYVYDFPELFRQASSSQWKNFSADVKLTDDFFISNELIEDENGELTEVEREPGANAIGMVAFKITVKTPEYPRGRQFVVVANDITFKIGSFGPQEDEFFNKVTEYARKRGIPRIYLAANSGARIGMAEEIVPLFQVAWNDAANPDKGFQYLYLTSEGMETLKKFDKENSVLTERTVINGEERFVIKTIIGSEDGLGVECLRGSGLIAGATSRAYHDIFTITLVTCRSVGIGAYLVRLGQRAIQVEGQPIILTGAPAINKMLGREVYTSNLQLGGTQIMYNNGVSHLTAVDDLAGVEKIVEWMSYVPAKRNMPVPILETKDTWDRPVDFTPTNDETYDVRWMIEGRETESGFEYGLFDKGSFFETLSGWAKGVVVGRARLGGIPLGVIGVETRTVENLIPADPANPNSAETLIQEPGQVWHPNSAFKTAQAINDFNNGEQLPMMILANWRGFSGGQRDMFNEVLKYGSFIVDALVDYKQPIIIYIPPTGELRGGSWVVVDPTINADQMEMYADVNARAGVLEPQGMVGIKFRREKLLDTMNRLDDKYRELRSQLSNKSLAPEVHQQISKQLADRERELLPIYGQISLQFADLHDRSSRMVAKGVISKELEWTEARRFFFWRLRRRLNEEYLIKRLSHQVGEASRLEKIARIRSWYPASVDHEDDRQVATWIEENYKTLDDKLKGLKLESFAQDLAKKIRSDHDNAIDGLSEVIKMLSTDDKEKLLKTLK

SEQ ID NO: 8 - protein, 2233 aa, Saccharomyces cerevisiae
MSEESLFESSPQKMEYEITNYSERHTELPGHFIGLNTVDKLEESPLRDFVKSHGGHTVISKILIANNGIAAVKEIRSVRKWAYETFGDDRTVQFVAMATPEDLEANAEYIRMADQYIEVPGGTNNNNYANVDLIVDIAERADVDAVWAGWGHASENPLLPEKLSQSKRKVIFIGPPGNAMRSLGDKISSTIVAQSAKVPCIPWSGTGVDTVHVDEKTGLVSVDDDIYQKGCCTSPEDGLQKAKRIGFPVMIKASEGGGGKGIRQVEREEDFIALYHQAANEIPGSPIFIMKLAGRARHLEVQLLADQYGTNISLFGRDCSVQRRHQKIIEEAPVTIAKAETFHEMEKAAVRLGKLVGYVSAGTVEYLYSHDDGKFYFLELNPRLQVEHPTTEMVSGVNLPAAQLQIAMGIPMHRISDIRTLYGMNPHSASEIDFEFKTQDATKKQRRPIPKGHCTACRITSEDPNDGFKPSGGTLHELNFRSSSNVWGYFSVGNNGNIHSFSDSQFGHIFAFGENRQASRKHMVVALKELSIRGDFRTTVEYLIKLLETEDFEDNTITTGWLDDLITHKMTAEKPDPTLAVICGAATKAFLASEEARHKYIESLQKGQVLSKDLLQTMFPVDFIHEGKRYKFTVAKSGNDRYTLFINGSKCDIILRQLVDGGLLIAIGGKSHTIYWKEEVAATRLSVDSMTTLLEVENDPTQLRTPSPGKLVKFLVENGEHIIKGQPYAEIEVMKMQMPLVSQENGIVQLLKQPGSTIVAGDIMAIMTLDDPSKVKHALPFEGMLPDFGSPVIEGTKPAYKFKSLVSTLENILKGYDNQVIMNASLQQLIEVLRNPKLPYSEWKLHISALHSRLPAKLDEQMEELVARSLRRGAVFPARQLSKLIDMAVKNPEYNPDKLLGAVVEPLADIAHKYSNGLEAHEHSIFVHFLEEYYEVEKLFNGPNVREENIILKLRDENPKDLDKVALTVLSHSKVSAKNNLILAILKHYQPLCKLSSKVSAIFSTPLQHIVELESKATAKVALQAREILIQGALPSVKERTEQIEHILKSSVVKVAYGSSNPKRSEPDLNILKDLIDSNYVVFDVLLQFLTHQDPVVTAAAAQVYIRRAYRAYTIGDIRVHEGVTVPIVEWKFQLPSAAFSTFPTVKSKMGMNRAVSVSDLSYVANSQSSPLREGILMAVDHLDDVDEILSQSLEVIPRHQSSSNGPAPDRSGSSASLSNVANVCVASTEGFESEEEILVRLREILDLNKQELINASIRRITFMFGFKDGSYPKYYTFNGPNYNENETIRHIEPALAFQLELGRLSNFNIKPIFTDNRNIHVYEAVSKTSPLDKRFFTRGIIRTGHIRDDISIQEYLTSEANRLMSDILDNLEVTDTSNSDLNHIFINFIAVFDISPEDVEAAFGGFLERFGKRLLRLRVSSAEIRIIIKDPQTGAPVPLRALINNVSGYVIKTEMYTEVKNAKGEWVFKSLGKPGSMHLRPIATPYPVKEWLQPKRYKAHLMGTTYVYDFPELFRQASSSQWKNFSADVKLTDDFFISNELIEDENGELTEVEREPGANAIGMVAFKITVKTPEYPRGRQFVVVANDITFKIGSFGPQEDEFFNKVTEYARKRGIPRIYLAANSGARIGMAEEIVPLFQVAWNDAANPDKGFQYLYLTSEGMETLKKFDKENSVLTERTVINGEERFVIKTIIGSEDGLGVECLRGSGLIAGATSRAYHDIFTITLVTCRSVGIGAYLVRLGQRAIQVEGQPIILTGAPAINKMLGREVYTSNLQLGGTQIMYNNGVSHLTAVDDLAGVEKIVEWMSYVPAKRNMPVPILETKDTWDRPVDFTPTNDETYDVRWMIEGRETESGFEYGLFDKGSFFETLSGWAKGVVVGRARLGGIPLGVIGVETRTVENLIPADPANPNSAETLIQEPGQVWHPNSAFKTAQAINDFNNGEQLPMMILANWRGFSGGQRDMFNEVLKYGSFIVDALVDYKQPIIIYIPPTGELRGGSWVVVDPTINADQMEMYADVNARAGVLEPQGMVGIKFRREKLLDTMNRLDDKYRELRSQLSNKSLAPEVHQQISKQLADRERELLPIYGQISLQFADLHDRSSRMVAKGVISKELEWTEARRFFFWRLRRRLNEEYLIKRLSHQVGEASRLEKIARIRSWYPASVDHEDDRQVATWIEENYKTLDDKLKGLKLESFAQDLAKKIRSDHDNAIDGLSEVIKMLSTDDKEKLLKTLK

SEQ ID NO: 9 - protein, 2233 aa, Saccharomyces cerevisiae
MSEESLFESSPQKMEYEITNYSERHTELPGHFIGLNTVDKLEESPLRDFVKSHGGHTVISKILIANNGIAAVKEIRSVRKWAYETFGDDRTVQFVAMATPEDLEANAEYIRMADQYIEVPGGTNNNNYANVDLIVDIAERADVDAVWAGWGHASENPLLPEKLSQSKRKVIFIGPPGNAMRSLGDKISSTIVAQSAKVPCIPWSGTGVDTVHVDEKTGLVSVDDDIYQKGCCTSPEDGLQKAKRIGFPVMIKASEGGGGKGIRQVEREEDFIALYHQAANEIPGSPIFIMKLAGRARHLEVQLLADQYGTNISLFGRDCSVQRRHQKIIEEAPVTIAKAETFHEMEKAAVRLGKLVGYVSAGTVEYLYSHDDGKFYFLELNPRLQVEHPTTEMVSGVNLPAAQLQIAMGIPMHRISDIRTLYGMNPHSASEIDFEFKTQDATKKQRRPIPKGHCTACRITSEDPNDGFKPSGGTLHELNFRSSSNVWGYFSVGNNGNIHSFSDSQFGHIFAFGENRQASRKHMVVALKELSIRGDFRTTVEYLIKLLETEDFEDNTITTGWLDDLITHKMTAEKPDPTLAVICGAATKAFLASEEARHKYIESLQKGQVLSKDLLQTMFPVDFIHEGKRYKFTVAKSGNDRYTLFINGSKCDIILRQLSDGGLLIAIGGKSHTIYWKEEVAATRLSVDSMTTLLEVENDPTQLRTPSPGKLVKFLVENGEHIIKGQPYAEIEVMKMQMPLVSQENGIVQLLKQPGSTIVAGDIMAIMTLDDPSKVKHALPFEGMLPDFGSPVIEGTKPAYKFKSLVSTLENILKGYDNQVIMNASLQQLIEVLRNPKLPYSEWKLHISALHSRLPAKLDEQMEELVARSLRRGAVFPARQLSKLIDMAVKNPEYNPDKLLGAVVEPLADIAHKYSNGLEAHEHSIFVHFLEEYYEVEKLFNGPNVREENIILKLRDENPKDLDKVALTVLSHSKVSAKNNLILAILKHYQPLCKLSSKVSAIFSTPLQHIVELESKATAKVALQAREILIQGALPSVKERTEQIEHILKSSVVKVAYGSSNPKRSEPDLNILKDLIDSNYVVFDVLLQFLTHQDPVVTAAAAQVYIRRAYRAYTIGDIRVHEGVTVPIVEWKFQLPSAAFSTFPTVKSKMGMNRAVAVSDLSYVANSQSSPLREGILMAVDHLDDVDEILSQSLEVIPRHQSSSNGPAPDRSGSSASLSNVANVCVASTEGFESEEEILVRLREILDLNKQELINASIRRITFMFGFKDGSYPKYYTFNGPNYNENETIRHIEPALAFQLELGRLSNFNIKPIFTDNRNIHVYEAVSKTSPLDKRFFTRGIIRTGHIRDDISIQEYLTSEANRLMSDILDNLEVTDTSNSDLNHIFINFIAVFDISPEDVEAAFGGFLERFGKRLLRLRVSSAEIRIIIKDPQTGAPVPLRALINNVSGYVIKTEMYTEVKNAKGEWVFKSLGKPGSMHLRPIATPYPVKEWLQPKRYKAHLMGTTYVYDFPELFRQASSSQWKNFSADVKLTDDFFISNELIEDENGELTEVEREPGANAIGMVAFKITVKTPEYPRGRQFVVVANDITFKIGSFGPQEDEFFNKVTEYARKRGIPRIYLAANSGARIGMAEEIVPLFQVAWNDAANPDKGFQYLYLTSEGMETLKKFDKENSVLTERTVINGEERFVIKTIIGSEDGLGVECLRGSGLIAGATSRAYHDIFTITLVTCRSVGIGAYLVRLGQRAIQVEGQPIILTGAPAINKMLGREVYTSNLQLGGTQIMYNNGVSHLTAVDDLAGVEKIVEWMSYVPAKRNMPVPILETKDTWDRPVDFTPTNDETYDVRWMIEGRETESGFEYGLFDKGSFFETLSGWAKGVVVGRARLGGIPLGVIGVETRTVENLIPADPANPNSAETLIQEPGQVWHPNSAFKTAQAINDFNNGEQLPMMILANWRGFSGGQRDMFNEVLKYGSFIVDALVDYKQPIIIYIPPTGELRGGSWVVVDPTINADQMEMYADVNARAGVLEPQGMVGIKFRREKLLDTMNRLDDKYRELRSQLSNKSLAPEVHQQISKQLADRERELLPIYGQISLQFADLHDRSSRMVAKGVISKELEWTEARRFFFWRLRRRLNEEYLIKRLSHQVGEASRLEKIARIRSWYPASVDHEDDRQVATWIEENYKTLDDKLKGLKLESFAQDLAKKIRSDHDNAIDGLSEVIKMLSTDDKEKLLKTLK

SEQ ID NO: 10 - protein, 2233 aa, Saccharomyces cerevisiae
MSEESLFESSPQKMEYEITNYSERHTELPGHFIGLNTVDKLEESPLRDFVKSHGGHTVISKILIANNGIAAVKEIRSVRKWAYETFGDDRTVQFVAMATPEDLEANAEYIRMADQYIEVPGGTNNNNYANVDLIVDIAERADVDAVWAGWGHASENPLLPEKLSQSKRKVIFIGPPGNAMRSLGDKISSTIVAQSAKVPCIPWSGTGVDTVHVDEKTGLVSVDDDIYQKGCCTSPEDGLQKAKRIGFPVMIKASEGGGGKGIRQVEREEDFIALYHQAANEIPGSPIFIMKLAGRARHLEVQLLADQYGTNISLFGRDCSVQRRHQKIIEEAPVTIAKAETFHEMEKAAVRLGKLVGYVSAGTVEYLYSHDDGKFYFLELNPRLQVEHPTTEMVSGVNLPAAQLQIAMGIPMHRISDIRTLYGMNPHSASEIDFEFKTQDATKKQRRPIPKGHCTACRITSEDPNDGFKPSGGTLHELNFRSSSNVWGYFSVGNNGNIHSFSDSQFGHIFAFGENRQASRKHMVVALKELSIRGDFRTTVEYLIKLLETEDFEDNTITTGWLDDLITHKMTAEKPDPTLAVICGAATKAFLASEEARHKYIESLQKGQVLSKDLLQTMFPVDFIHEGKRYKFTVAKSGNDRYTLFINGSKCDIILRQLSDGGLLIAIGGKSHTIYWKEEVAATRLSVDSMTTLLEVENDPTQLRTPSPGKLVKFLVENGEHIIKGQPYAEIEVMKMQMPLVSQENGIVQLLKQPGSTIVAGDIMAIMTLDDPSKVKHALPFEGMLPDFGSPVIEGTKPAYKFKSLVSTLENILKGYDNQVIMNASLQQLIEVLRNPKLPYSEWKLHISALHSRLPAKLDEQMEELVARSLRRGAVFPARQLSKLIDMAVKNPEYNPDKLLGAVVEPLADIAHKYSNGLEAHEHSIFVHFLEEYYEVEKLFNGPNVREENIILKLRDENPKDLDKVALTVLSHSKVSAKNNLILAILKHYQPLCKLSSKVSAIFSTPLQHIVELESKATAKVALQAREILIQGALPSVKERTEQIEHILKSSVVKVAYGSSNPKRSEPDLNILKDLIDSNYVVFDVLLQFLTHQDPVVTAAAAQVYIRRAYRAYTIGDIRVHEGVTVPIVEWKFQLPSAAFSTFPTVKSKMGMNRAVVVSDLSYVANSQSSPLREGILMAVDHLDDVDEILSQSLEVIPRHQSSSNGPAPDRSGSSASLSNVANVCVASTEGFESEEEILVRLREILDLNKQELINASIRRITFMFGFKDGSYPKYYTFNGPNYNENETIRHIEPALAFQLELGRLSNFNIKPIFTDNRNIHVYEAVSKTSPLDKRFFTRGIIRTGHIRDDISIQEYLTSEANRLMSDILDNLEVTDTSNSDLNHIFINFIAVFDISPEDVEAAFGGFLERFGKRLLRLRVSSAEIRIIIKDPQTGAPVPLRALINNVSGYVIKTEMYTEVKNAKGEWVFKSLGKPGSMHLRPIATPYPVKEWLQPKRYKAHLMGTTYVYDFPELFRQASSSQWKNFSADVKLTDDFFISNELIEDENGELTEVEREPGANAIGMVAFKITVKTPEYPRGRQFVVVANDITFKIGSFGPQEDEFFNKVTEYARKRGIPRIYLAANSGARIGMAEEIVPLFQVAWNDAANPDKGFQYLYLTSEGMETLKKFDKENSVLTERTVINGEERFVIKTIIGSEDGLGVECLRGSGLIAGATSRAYHDIFTITLVTCRSVGIGAYLVRLGQRAIQVEGQPIILTGAPAINKMLGREVYTSNLQLGGTQIMYNNGVSHLTAVDDLAGVEKIVEWMSYVPAKRNMPVPILETKDTWDRPVDFTPTNDETYDVRWMIEGRETESGFEYGLFDKGSFFETLSGWAKGVVVGRARLGGIPLGVIGVETRTVENLIPADPANPNSAETLIQEPGQVWHPNSAFKTAQAINDFNNGEQLPMMILANWRGFSGGQRDMFNEVLKYGSFIVDALVDYKQPIIIYIPPTGELRGGSWVVVDPTINADQMEMYADVNARAGVLEPQGMVGIKFRREKLLDTMNRLDDKYRELRSQLSNKSLAPEVHQQISKQLADRERELLPIYGQISLQFADLHDRSSRMVAKGVISKELEWTEARRFFFWRLRRRLNEEYLIKRLSHQVGEASRLEKIARIRSWYPASVDHEDDRQVATWIEENYKTLDDKLKGLKLESFAQDLAKKIRSDHDNAIDGLSEVIKMLSTDDKEKLLKTLK

SEQ ID NO: 11 - protein, 2233 aa, Saccharomyces cerevisiae
MSEESLFESSPQKMEYEITNYSERHTELPGHFIGLNTVDKLEESPLRDFVKSHGGHTVISKILIANNGIAAVKEIRSVRKWAYETFGDDRTVQFVAMATPEDLEANAEYIRMADQYIEVPGGTNNNNYANVDLIVDIAERADVDAVWAGWGHASENPLLPEKLSQSKRKVIFIGPPGNAMRSLGDKISSTIVAQSAKVPCIPWSGTGVDTVHVDEKTGLVSVDDDIYQKGCCTSPEDGLQKAKRIGFPVMIKASEGGGGKGIRQVEREEDFIALYHQAANEIPGSPIFIMKLAGRARHLEVQLLADQYGTNISLFGRDCSVQRRHQKIIEEAPVTIAKAETFHEMEKAAVRLGKLVGYVSAGTVEYLYSHDDGKFYFLELNPRLQVEHPTTEMVSGVNLPAAQLQIAMGIPMHRISDIRTLYGMNPHSASEIDFEFKTQDATKKQRRPIPKGHCTACRITSEDPNDGFKPSGGTLHELNFRSSSNVWGYFSVGNNGNIHSFSDSQFGHIFAFGENRQASRKHMVVALKELSIRGDFRTTVEYLIKLLETEDFEDNTITTGWLDDLITHKMTAEKPDPTLAVICGAATKAFLASEEARHKYIESLQKGQVLSKDLLQTMFPVDFIHEGKRYKFTVAKSGNDRYTLFINGSKCDIILRQLADGGLLIAIGGKSHTIYWKEEVAATRLSVDSMTTLLEVENDPTQLRTPSPGKLVKFLVENGEHIIKGQPYAEIEVMKMQMPLVSQENGIVQLLKQPGSTIVAGDIMAIMTLDDPSKVKHALPFEGMLPDFGSPVIEGTKPAYKFKSLVSTLENILKGYDNQVIMNASLQQLIEVLRNPKLPYSEWKLHISALHSRLPAKLDEQMEELVARSLRRGAVFPARQLSKLIDMAVKNPEYNPDKLLGAVVEPLADIAHKYSNGLEAHEHSIFVHFLEEYYEVEKLFNGPNVREENIILKLRDENPKDLDKVALTVLSHSKVSAKNNLILAILKHYQPLCKLSSKVSAIFSTPLQHIVELESKATAKVALQAREILIQGALPSVKERTEQIEHILKSSVVKVAYGSSNPKRSEPDLNILKDLIDSNYVVFDVLLQFLTHQDPVVTAAAAQVYIRRAYRAYTIGDIRVHEGVTVPIVEWKFQLPSAAFSTFPTVKSKMGMNRAVAVSDLSYVANSQSSPLREGILMAVDHLDDVDEILSQSLEVIPRHQSSSNGPAPDRSGSSASLSNVANVCVASTEGFESEEEILVRLREILDLNKQELINASIRRITFMFGFKDGSYPKYYTFNGPNYNENETIRHIEPALAFQLELGRLSNFNIKPIFTDNRNIHVYEAVSKTSPLDKRFFTRGIIRTGHIRDDISIQEYLTSEANRLMSDILDNLEVTDTSNSDLNHIFINFIAVFDISPEDVEAAFGGFLERFGKRLLRLRVSSAEIRIIIKDPQTGAPVPLRALINNVSGYVIKTEMYTEVKNAKGEWVFKSLGKPGSMHLRPIATPYPVKEWLQPKRYKAHLMGTTYVYDFPELFRQASSSQWKNFSADVKLTDDFFISNELIEDENGELTEVEREPGANAIGMVAFKITVKTPEYPRGRQFVVVANDITFKIGSFGPQEDEFFNKVTEYARKRGIPRIYLAANSGARIGMAEEIVPLFQVAWNDAANPDKGFQYLYLTSEGMETLKKFDKENSVLTERTVINGEERFVIKTIIGSEDGLGVECLRGSGLIAGATSRAYHDIFTITLVTCRSVGIGAYLVRLGQRAIQVEGQPIILTGAPAINKMLGREVYTSNLQLGGTQIMYNNGVSHLTAVDDLAGVEKIVEWMSYVPAKRNMPVPILETKDTWDRPVDFTPTNDETYDVRWMIEGRETESGFEYGLFDKGSFFETLSGWAKGVVVGRARLGGIPLGVIGVETRTVENLIPADPANPNSAETLIQEPGQVWHPNSAFKTAQAINDFNNGEQLPMMILANWRGFSGGQRDMFNEVLKYGSFIVDALVDYKQPIIIYIPPTGELRGGSWVVVDPTINADQMEMYADVNARAGVLEPQGMVGIKFRREKLLDTMNRLDDKYRELRSQLSNKSLAPEVHQQISKQLADRERELLPIYGQISLQFADLHDRSSRMVAKGVISKELEWTEARRFFFWRLRRRLNEEYLIKRLSHQVGEASRLEKIARIRSWYPASVDHEDDRQVATWIEENYKTLDDKLKGLKLESFAQDLAKKIRSDHDNAIDGLSEVIKMLSTDDKEKLLKTLK

SEQ ID NO: 12 - protein, 2233 aa, Saccharomyces cerevisiae
MSEESLFESSPQKMEYEITNYSERHTELPGHFIGLNTVDKLEESPLRDFVKSHGGHTVISKILIANNGIAAVKEIRSVRKWAYETFGDDRTVQFVAMATPEDLEANAEYIRMADQYIEVPGGTNNNNYANVDLIVDIAERADVDAVWAGWGHASENPLLPEKLSQSKRKVIFIGPPGNAMRSLGDKISSTIVAQSAKVPCIPWSGTGVDTVHVDEKTGLVSVDDDIYQKGCCTSPEDGLQKAKRIGFPVMIKASEGGGGKGIRQVEREEDFIALYHQAANEIPGSPIFIMKLAGRARHLEVQLLADQYGTNISLFGRDCSVQRRHQKIIEEAPVTIAKAETFHEMEKAAVRLGKLVGYVSAGTVEYLYSHDDGKFYFLELNPRLQVEHPTTEMVSGVNLPAAQLQIAMGIPMHRISDIRTLYGMNPHSASEIDFEFKTQDATKKQRRPIPKGHCTACRITSEDPNDGFKPSGGTLHELNFRSSSNVWGYFSVGNNGNIHSFSDSQFGHIFAFGENRQASRKHMVVALKELSIRGDFRTTVEYLIKLLETEDFEDNTITTGWLDDLITHKMTAEKPDPTLAVICGAATKAFLASEEARHKYIESLQKGQVLSKDLLQTMFPVDFIHEGKRYKFTVAKSGNDRYTLFINGSKCDIILRQLADGGLLIAIGGKSHTIYWKEEVAATRLSVDSMTTLLEVENDPTQLRTPSPGKLVKFLVENGEHIIKGQPYAEIEVMKMQMPLVSQENGIVQLLKQPGSTIVAGDIMAIMTLDDPSKVKHALPFEGMLPDFGSPVIEGTKPAYKFKSLVSTLENILKGYDNQVIMNASLQQLIEVLRNPKLPYSEWKLHISALHSRLPAKLDEQMEELVARSLRRGAVFPARQLSKLIDMAVKNPEYNPDKLLGAVVEPLADIAHKYSNGLEAHEHSIFVHFLEEYYEVEKLFNGPNVREENIILKLRDENPKDLDKVALTVLSHSKVSAKNNLILAILKHYQPLCKLSSKVSAIFSTPLQHIVELESKATAKVALQAREILIQGALPSVKERTEQIEHILKSSVVKVAYGSSNPKRSEPDLNILKDLIDSNYVVFDVLLQFLTHQDPVVTAAAAQVYIRRAYRAYTIGDIRVHEGVTVPIVEWKFQLPSAAFSTFPTVKSKMGMNRAVVVSDLSYVANSQSSPLREGILMAVDHLDDVDEILSQSLEVIPRHQSSSNGPAPDRSGSSASLSNVANVCVASTEGFESEEEILVRLREILDLNKQELINASIRRITFMFGFKDGSYPKYYTFNGPNYNENETIRHIEPALAFQLELGRLSNFNIKPIFTDNRNIHVYEAVSKTSPLDKRFFTRGIIRTGHIRDDISIQEYLTSEANRLMSDILDNLEVTDTSNSDLNHIFINFIAVFDISPEDVEAAFGGFLERFGKRLLRLRVSSAEIRIIIKDPQTGAPVPLRALINNVSGYVIKTEMYTEVKNAKGEWVFKSLGKPGSMHLRPIATPYPVKEWLQPKRYKAHLMGTTYVYDFPELFRQASSSQWKNFSADVKLTDDFFISNELIEDENGELTEVEREPGANAIGMVAFKITVKTPEYPRGRQFVVVANDITFKIGSFGPQEDEFFNKVTEYARKRGIPRIYLAANSGARIGMAEEIVPLFQVAWNDAANPDKGFQYLYLTSEGMETLKKFDKENSVLTERTVINGEERFVIKTIIGSEDGLGVECLRGSGLIAGATSRAYHDIFTITLVTCRSVGIGAYLVRLGQRAIQVEGQPIILTGAPAINKMLGREVYTSNLQLGGTQIMYNNGVSHLTAVDDLAGVEKIVEWMSYVPAKRNMPVPILETKDTWDRPVDFTPTNDETYDVRWMIEGRETESGFEYGLFDKGSFFETLSGWAKGVVVGRARLGGIPLGVIGVETRTVENLIPADPANPNSAETLIQEPGQVWHPNSAFKTAQAINDFNNGEQLPMMILANWRGFSGGQRDMFNEVLKYGSFIVDALVDYKQPIIIYIPPTGELRGGSWVVVDPTINADQMEMYADVNARAGVLEPQGMVGIKFRREKLLDTMNRLDDKYRELRSQLSNKSLAPEVHQQISKQLADRERELLPIYGQISLQFADLHDRSSRMVAKGVISKELEWTEARRFFFWRLRRRLNEEYLIKRLSHQVGEASRLEKIARIRSWYPASVDHEDDRQVATWIEENYKTLDDKLKGLKLESFAQDLAKKIRSDHDNAIDGLSEVIKMLSTDDKEKLLKTLK

SEQ ID NO: 13 - protein, 2233 aa, Saccharomyces cerevisiae
MSEESLFESSPQKMEYEITNYSERHTELPGHFIGLNTVDKLEESPLRDFVKSHGGHTVISKILIANNGIAAVKEIRSVRKWAYETFGDDRTVQFVAMATPEDLEANAEYIRMADQYIEVPGGTNNNNYANVDLIVDIAERADVDAVWAGWGHASENPLLPEKLSQSKRKVIFIGPPGNAMRSLGDKISSTIVAQSAKVPCIPWSGTGVDTVHVDEKTGLVSVDDDIYQKGCCTSPEDGLQKAKRIGFPVMIKASEGGGGKGIRQVEREEDFIALYHQAANEIPGSPIFIMKLAGRARHLEVQLLADQYGTNISLFGRDCSVQRRHQKIIEEAPVTIAKAETFHEMEKAAVRLGKLVGYVSAGTVEYLYSHDDGKFYFLELNPRLQVEHPTTEMVSGVNLPAAQLQIAMGIPMHRISDIRTLYGMNPHSASEIDFEFKTQDATKKQRRPIPKGHCTACRITSEDPNDGFKPSGGTLHELNFRSSSNVWGYFSVGNNGNIHSFSDSQFGHIFAFGENRQASRKHMVVALKELSIRGDFRTTVEYLIKLLETEDFEDNTITTGWLDDLITHKMTAEKPDPTLAVICGAATKAFLASEEARHKYIESLQKGQVLSKDLLQTMFPVDFIHEGKRYKFTVAKSGNDRYTLFINGSKCDIILRQLVDGGLLIAIGGKSHTIYWKEEVAATRLSVDSMTTLLEVENDPTQLRTPSPGKLVKFLVENGEHIIKGQPYAEIEVMKMQMPLVSQENGIVQLLKQPGSTIVAGDIMAIMTLDDPSKVKHALPFEGMLPDFGSPVIEGTKPAYKFKSLVSTLENILKGYDNQVIMNASLQQLIEVLRNPKLPYSEWKLHISALHSRLPAKLDEQMEELVARSLRRGAVFPARQLSKLIDMAVKNPEYNPDKLLGAVVEPLADIAHKYSNGLEAHEHSIFVHFLEEYYEVEKLFNGPNVREENIILKLRDENPKDLDKVALTVLSHSKVSAKNNLILAILKHYQPLCKLSSKVSAIFSTPLQHIVELESKATAKVALQAREILIQGALPSVKERTEQIEHILKSSVVKVAYGSSNPKRSEPDLNILKDLIDSNYVVFDVLLQFLTHQDPVVTAAAAQVYIRRAYRAYTIGDIRVHEGVTVPIVEWKFQLPSAAFSTFPTVKSKMGMNRAVAVSDLSYVANSQSSPLREGILMAVDHLDDVDEILSQSLEVIPRHQSSSNGPAPDRSGSSASLSNVANVCVASTEGFESEEEILVRLREILDLNKQELINASIRRITFMFGFKDGSYPKYYTFNGPNYNENETIRHIEPALAFQLELGRLSNFNIKPIFTDNRNIHVYEAVSKTSPLDKRFFTRGIIRTGHIRDDISIQEYLTSEANRLMSDILDNLEVTDTSNSDLNHIFINFIAVFDISPEDVEAAFGGFLERFGKRLLRLRVSSAEIRIIIKDPQTGAPVPLRALINNVSGYVIKTEMYTEVKNAKGEWVFKSLGKPGSMHLRPIATPYPVKEWLQPKRYKAHLMGTTYVYDFPELFRQASSSQWKNFSADVKLTDDFFISNELIEDENGELTEVEREPGANAIGMVAFKITVKTPEYPRGRQFVVVANDITFKIGSFGPQEDEFFNKVTEYARKRGIPRIYLAANSGARIGMAEEIVPLFQVAWNDAANPDKGFQYLYLTSEGMETLKKFDKENSVLTERTVINGEERFVIKTIIGSEDGLGVECLRGSGLIAGATSRAYHDIFTITLVTCRSVGIGAYLVRLGQRAIQVEGQPIILTGAPAINKMLGREVYTSNLQLGGTQIMYNNGVSHLTAVDDLAGVEKIVEWMSYVPAKRNMPVPILETKDTWDRPVDFTPTNDETYDVRWMIEGRETESGFEYGLFDKGSFFETLSGWAKGVVVGRARLGGIPLGVIGVETRTVENLIPADPANPNSAETLIQEPGQVWHPNSAFKTAQAINDFNNGEQLPMMILANWRGFSGGQRDMFNEVLKYGSFIVDALVDYKQPIIIYIPPTGELRGGSWVVVDPTINADQMEMYADVNARAGVLEPQGMVGIKFRREKLLDTMNRLDDKYRELRSQLSNKSLAPEVHQQISKQLADRERELLPIYGQISLQFADLHDRSSRMVAKGVISKELEWTEARRFFFWRLRRRLNEEYLIKRLSHQVGEASRLEKIARIRSWYPASVDHEDDRQVATWIEENYKTLDDKLKGLKLESFAQDLAKKIRSDHDNAIDGLSEVIKMLSTDDKEKLLKTLK

SEQ ID NO: 14 - protein, 2233 aa, Saccharomyces cerevisiae
MSEESLFESSPQKMEYEITNYSERHTELPGHFIGLNTVDKLEESPLRDFVKSHGGHTVISKILIANNGIAAVKEIRSVRKWAYETFGDDRTVQFVAMATPEDLEANAEYIRMADQYIEVPGGTNNNNYANVDLIVDIAERADVDAVWAGWGHASENPLLPEKLSQSKRKVIFIGPPGNAMRSLGDKISSTIVAQSAKVPCIPWSGTGVDTVHVDEKTGLVSVDDDIYQKGCCTSPEDGLQKAKRIGFPVMIKASEGGGGKGIRQVEREEDFIALYHQAANEIPGSPIFIMKLAGRARHLEVQLLADQYGTNISLFGRDCSVQRRHQKIIEEAPVTIAKAETFHEMEKAAVRLGKLVGYVSAGTVEYLYSHDDGKFYFLELNPRLQVEHPTTEMVSGVNLPAAQLQIAMGIPMHRISDIRTLYGMNPHSASEIDFEFKTQDATKKQRRPIPKGHCTACRITSEDPNDGFKPSGGTLHELNFRSSSNVWGYFSVGNNGNIHSFSDSQFGHIFAFGENRQASRKHMVVALKELSIRGDFRTTVEYLIKLLETEDFEDNTITTGWLDDLITHKMTAEKPDPTLAVICGAATKAFLASEEARHKYIESLQKGQVLSKDLLQTMFPVDFIHEGKRYKFTVAKSGNDRYTLFINGSKCDIILRQLVDGGLLIAIGGKSHTIYWKEEVAATRLSVDSMTTLLEVENDPTQLRTPSPGKLVKFLVENGEHIIKGQPYAEIEVMKMQMPLVSQENGIVQLLKQPGSTIVAGDIMAIMTLDDPSKVKHALPFEGMLPDFGSPVIEGTKPAYKFKSLVSTLENILKGYDNQVIMNASLQQLIEVLRNPKLPYSEWKLHISALHSRLPAKLDEQMEELVARSLRRGAVFPARQLSKLIDMAVKNPEYNPDKLLGAVVEPLADIAHKYSNGLEAHEHSIFVHFLEEYYEVEKLFNGPNVREENIILKLRDENPKDLDKVALTVLSHSKVSAKNNLILAILKHYQPLCKLSSKVSAIFSTPLQHIVELESKATAKVALQAREILIQGALPSVKERTEQIEHILKSSVVKVAYGSSNPKRSEPDLNILKDLIDSNYVVFDVLLQFLTHQDPVVTAAAAQVYIRRAYRAYTIGDIRVHEGVTVPIVEWKFQLPSAAFSTFPTVKSKMGMNRAVVVSDLSYVANSQSSPLREGILMAVDHLDDVDEILSQSLEVIPRHQSSSNGPAPDRSGSSASLSNVANVCVASTEGFESEEEILVRLREILDLNKQELINASIRRITFMFGFKDGSYPKYYTFNGPNYNENETIRHIEPALAFQLELGRLSNFNIKPIFTDNRNIHVYEAVSKTSPLDKRFFTRGIIRTGHIRDDISIQEYLTSEANRLMSDILDNLEVTDTSNSDLNHIFINFIAVFDISPEDVEAAFGGFLERFGKRLLRLRVSSAEIRIIIKDPQTGAPVPLRALINNVSGYVIKTEMYTEVKNAKGEWVFKSLGKPGSMHLRPIATPYPVKEWLQPKRYKAHLMGTTYVYDFPELFRQASSSQWKNFSADVKLTDDFFISNELIEDENGELTEVEREPGANAIGMVAFKITVKTPEYPRGRQFVVVANDITFKIGSFGPQEDEFFNKVTEYARKRGIPRIYLAANSGARIGMAEEIVPLFQVAWNDAANPDKGFQYLYLTSEGMETLKKFDKENSVLTERTVINGEERFVIKTIIGSEDGLGVECLRGSGLIAGATSRAYHDIFTITLVTCRSVGIGAYLVRLGQRAIQVEGQPIILTGAPAINKMLGREVYTSNLQLGGTQIMYNNGVSHLTAVDDLAGVEKIVEWMSYVPAKRNMPVPILETKDTWDRPVDFTPTNDETYDVRWMIEGRETESGFEYGLFDKGSFFETLSGWAKGVVVGRARLGGIPLGVIGVETRTVENLIPADPANPNSAETLIQEPGQVWHPNSAFKTAQAINDFNNGEQLPMMILANWRGFSGGQRDMFNEVLKYGSFIVDALVDYKQPIIIYIPPTGELRGGSWVVVDPTINADQMEMYADVNARAGVLEPQGMVGIKFRREKLLDTMNRLDDKYRELRSQLSNKSLAPEVHQQISKQLADRERELLPIYGQISLQFADLHDRSSRMVAKGVISKELEWTEARRFFFWRLRRRLNEEYLIKRLSHQVGEASRLEKIARIRSWYPASVDHEDDRQVATWIEENYKTLDDKLKGLKLESFAQDLAKKIRSDHDNAIDGLSEVIKMLSTDDKEKLLKTLK

SEQ ID NO: 15 - protein, 256 aa, Saccharomyces cerevisiae
MDFTKPETVLNLQNIRDELVRMEDSIIFKFIERSHFATCPSVYEANHPGLEIPNFKGSFLDWALSNLEIAHSRIRRFESPDETPFFPDKIQKSFLPSINYPQILAPYAPEVNYNDKIKKVYIEKIIPLISKRDGDDKNNFGSVATRDIECLQSLSRRIHFGKFVAEAKFQSDIPLYTKLIKSKDVEGIMKNITNSAVEEKILERLTKKAEVYGVDPTNESGERRINPEYLVKIYKEIVIPITKEVEVEYLLRRLEE

SEQ ID NO: 16 - protein, 717 aa, Arabidopsis thaliana
MDQIEAMLCGGGEKTKVAVTTKTLADPLNWGLAADQMKGSHLDEVKKMVEEYRRPVVNLGGETLTIGQVAAISTVGGSVKVELAETSRAGVKASSDWVMESMNKGTDSYGVTTGFGATSHRRTKNGTALQTELIRFLNAGIFGNTKETCHTLPQSATRAAMLVRVNTLLQGYSGIRFEILEAITSLLNHNISPSLPLRGTITASGDLVPLSYIAGLLTGRPNSKATGPDGESLTAKEAFEKAGISTGFFDLQPKEGLALVNGTAVGSGMASMVLFEANVQAVLAEVLSAIFAEVMSGKPEFTDHLTHRLKHHPGQIEAAAIMEHILDGSSYMKLAQKVHEMDPLQKPKQDRYALRTSPQWLGPQIEVIRQATKSIEREINSVNDNPLIDVSRNKAIHGGNFQGTPIGVSMDNTRLAIAAIGKLMFAQFSELVNDFYNNGLPSNLTASSNPSLDYGFKGAEIAMASYCSELQYLANPVTSHVQSAEQHNQDVNSLGLISSRKTSEAVDILKLMSTTFLVGICQAVDLRHLEENLRQTVKNTVSQVAKKVLTTGINGELHPSRFCEKDLLKVVDREQVFTYVDDPCSATYPLMQRLRQVIVDHALSNGETEKNAVTSIFQKIGAFEEELKAVLPKEVEAARAAYGNGTAPIPNRIKECRSYPLYRFVREELGTKLLTGEKVVSPGEEFDKVFTAMCEGKLIDPLMDCLKEWNGAPIPIC

SEQ ID NO: 17 - protein, 531 aa, Rhodobacter capsulatus
MTLQSQTAKDCLALDGALTLVQCEAIATHRSRISVTPALRERCARAHARLEHAIAEQRHIYGITTGFGPLANRLIGADQGAELQQNLIYHLATGVGPKLSWAEARALMLARLNSILQGASGASPETIDRIVAVLNAGFAPEVPAQGTVGASGDLTPLAHMVLALQGRGRMIDPSGRVQEAGAVMDRLCGGPLTLAARDGLALVNGTSAMTAIAALTGVEAARAIDAALRHSAVLMEVLSGHAEAWHPAFAELRPHPGQLRATERLAQALDGAGRVCRTLTAARRLTAADLRPEDHPAQDAYSLRVVPQLVGAVWDTLDWHDRVVTCELNSVTDNPIFPEGCAVPALHGGNFMGVHVALASDALNAALVTLAGLVERQIARLTDEKLNKGLPAFLHGGQAGLQSGFMGAQVTATALLAEMRANATPVSVQSLSTNGANQDVVSMGTIAARRARAQLLPLSQIQAILALALAQAMDLLDDPEGQAGWSLTARDLRDRIRAVSPGLRADRPLAGHIEAVAQGLRHPSAAADPPA

SEQ ID NO: 18 - protein, 505 aa, Arabidopsis thaliana
MDLLLLEKSLIAVFVAVILATVISKLRGKKLKLPPGPIPIPIFGNWLQVGDDLNHRNLVDYAKKFGDLFLLRMGQRNLVVVSSPDLTKEVLLTQGVEFGSRTRNVVFDIFTGKGQDMVFTVYGEHWRKMRRIMTVPFFTNKVVQQNREGWEFEAASVVEDVKKNPDSATKGIVLRKRLQLMMYNNMFRIMFDRRFESEDDPLFLRLKALNGERSRLAQSFEYNYGDFIPILRPFLRGYLKICQDVKDRRIALFKKYFVDERKQIASSKPTGSEGLKCAIDHILEAEQKGEINEDNVLYIVENINVAAIETTLWSIEWGIAELVNHPEIQSKLRNELDTVLGPGVQVTEPDLHKLPYLQAVVKETLRLRMAIPLLVPHMNLHDAKLAGYDIPAESKILVNAWWLANNPNSWKKPEEFRPERFFEEESHVEANGNDFRYVPFGVGRRSCPGIILALPILGITIGRMVQNFELLPPPGQSKVDTSEKGGQFSLHILNHSIIVMKPRNC

SEQ ID NO: 19 - protein, 556 aa, Arabidopsis thaliana
MTTQDVIVNDQNDQKQCSNDVIFRSRLPDIYIPNHLPLHDYIFENISEFAAKPCLINGPTGEVYTYADVHVTSRKLAAGLHNLGVKQHDVVMILLPNSPEVVLTFLAASFIGAITTSANPFFTPAEISKQAKASAAKLIVTQSRYVDKIKNLQNDGVLIVTTDSDAIPENCLRFSELTQSEEPRVDSIPEKISPEDVVALPFSSGTTGLPKGVMLTHKGLVTSVAQQVDGENPNLYFNRDDVILCVLPMFHIYALNSIMLCSLRVGATILIMPKFEITLLLEQIQRCKVTVAMVVPPIVLAIAKSPETEKYDLSSVRMVKSGAAPLGKELEDAISAKFPNAKLGQGYGMTEAGPVLAMSLGFAKEPFPVKSGACGTVVRNAEMKILDPDTGDSLPRNKPGEICIRGNQIMKGYLNDPLATASTIDKDGWLHTGDVGFIDDDDELFIVDRLKELIKYKGFQVAPAELESLLIGHPEINDVAVVAMKEEDAGEVPVAFVVRSKDSNISEDEIKQFVSKQVVFYKRINKVFFTDSIPKAPSGKILRKDLRARLANGLMN

SEQ ID NO: 20 - protein, 392 aa, Vitus pseudoreticulata
MASVEEIRNAQRAKGPATILAIGTATPDHCVYQSDYADYYFRVTKSEHMTALKKKFNRICDKSMIKKRYIHLTEEMLEEHPNIGAYMAPSLNIRQEIITAEVPKLGKEAALKALKEWGQPKSKITHLVFCTTSGVEMPGADYKLANLLGLEPSVRRVMLYHQGCYAGGTVLRTTKDLAENNAGARVLVVCPEITVVTFRGPSEDALDSLVGQALFGDGSAAVIVGSDPDISIERPLFQLVSAAQTFIPNFAGAIAGNLREVGLTFHLWPNVPTLISENIENCLTQAFDPLGISDWNSLFWIAHPGGPAILDAVEAKLNLDKKKLEATRHVLSEYGNVSSACVLFILDEMRKKSLKGERATTGEGLGWGVLFGFGPGLTIETVVLHSIPMVTN

SEQ ID NO: 21 - protein, 711 aa, Arabidopsis thaliana
MSSSSSSSTSMIDLMAAIIKGEPVIVSDPANASAYESVAAELSSMLIENRQFAMIVTTSIAVLIGCIVMLVWRRSGSGNSKRVEPLKPLVIKPREEEIDDGRKKVTIFFGTQTGTAEGFAKALGEEAKARYEKTRFKIVDLDDYAADDDEYEEKLKKEDVAFFFLATYGDGEPTDNAARFYKWFTEGNDRGEWLKNLKYGVFGLGNRQYEHFNKVAKVVDDILVEQGAQRLVQVGLGDDDQCIEDDFTAWREALWPELDTILREEGDTAVATPYTAAVLEYRVSIHDSEDAKFNDINMANGNGYTVFDAQHPYKANVAVKRELHTPESDRSCIHLEFDIAGSGLTYETGDHVGVLCDNLSETVDEALRLLDMSPDTYFSLHAEKEDGTPISSSLPPPFPPCNLRTALTRYACLLSSPKKSALVALAAHASDPTEAERLKHLASPAGKDEYSKWVVESQRSLLEVMAEFPSAKPPLGVFFAGVAPRLQPRFYSISSSPKIAETRIHVTCALVYEKMPTGRIHKGVCSTWMKNAVPYEKSENCSSAPIFVRQSNFKLPSDSKVPIIMIGPGTGLAPFRGFLQERLALVESGVELGPSVLFFGCRNRRMDFIYEEELQRFVESGALAELSVAFSREGPTKEYVQHKMMDKASDIWNMISQGAYLYVCGDAKGMARDVHRSLHTIAQEQGSMDSTKAEGFVKNLQTSGRYLRDVW

SEQ ID NO: 22 - protein, 370 aa, Saccharomyces cerevisiae
MSESPMFAANGMPKVNQGAEEDVRILGYDPLASPALLQVQIPATPTSLETAKRGRREAIDIITGKDDRVLVIVGPCSIHDLEAAQEYALRLKKLSDELKGDLSIIMRAYLEKPRTTVGWKGLINDPDVNNTFNINKGLQSARQLFVNLTNIGLPIGSEMLDTISPQYLADLVSFGAIGARTTESQLHRELASGLSFPVGFKNGTDGTLNVAVDACQAAAHSHHFMGVTPHGVAAITTTKGNEHCFVILRGGKKGTNYDAKSVAEAKAQLPAGSNGLMIDYSHGNSNKDFRNQPKVNDVVCEQIANGENAITGVMIESNINEGNQGIPAEGKAGLKYGVSITDACIGWETTEDVLRKLAAAVRQRREVNKK

SEQ ID NO: 23 - protein, 2233 aa, Saccharomyces cerevisiae
MSEESLFESSPQKMEYEITNYSERHTELPGHFIGLNTVDKLEESPLRDFVKSHGGHTVISKILIANNGIAAVKEIRSVRKWAYETFGDDRTVQFVAMATPEDLEANAEYIRMADQYIEVPGGTNNNNYANVDLIVDIAERADVDAVWAGWGHASENPLLPEKLSQSKRKVIFIGPPGNAMRSLGDKISSTIVAQSAKVPCIPWSGTGVDTVHVDEKTGLVSVDDDIYQKGCCTSPEDGLQKAKRIGFPVMIKASEGGGGKGIRQVEREEDFIALYHQAANEIPGSPIFIMKLAGRARHLEVQLLADQYGTNISLFGRDCSVQRRHQKIIEEAPVTIAKAETFHEMEKAAVRLGKLVGYVSAGTVEYLYSHDDGKFYFLELNPRLQVEHPTTEMVSGVNLPAAQLQIAMGIPMHRISDIRTLYGMNPHSASEIDFEFKTQDATKKQRRPIPKGHCTACRITSEDPNDGFKPSGGTLHELNFRSSSNVWGYFSVGNNGNIHSFSDSQFGHIFAFGENRQASRKHMVVALKELSIRGDFRTTVEYLIKLLETEDFEDNTITTGWLDDLITHKMTAEKPDPTLAVICGAATKAFLASEEARHKYIESLQKGQVLSKDLLQTMFPVDFIHEGKRYKFTVAKSGNDRYTLFINGSKCDIILRQLPDGGLLIAIGGKSHTIYWKEEVAATRLSVDSMTTLLEVENDPTQLRTPSPGKLVKFLVENGEHIIKGQPYAEIEVMKMQMPLVSQENGIVQLLKQPGSTIVAGDIMAIMTLDDPSKVKHALPFEGMLPDFGSPVIEGTKPAYKFKSLVSTLENILKGYDNQVIMNASLQQLIEVLRNPKLPYSEWKLHISALHSRLPAKLDEQMEELVARSLRRGAVFPARQLSKLIDMAVKNPEYNPDKLLGAVVEPLADIAHKYSNGLEAHEHSIFVHFLEEYYEVEKLFNGPNVREENIILKLRDENPKDLDKVALTVLSHSKVSAKNNLILAILKHYQPLCKLSSKVSAIFSTPLQHIVELESKATAKVALQAREILIQGALPSVKERTEQIEHILKSSVVKVAYGSSNPKRSEPDLNILKDLIDSNYVVFDVLLQFLTHQDPVVTAAAAQVYIRRAYRAYTIGDIRVHEGVTVPIVEWKFQLPSAAFSTFPTVKSKMGMNRAVSVSDLSYVANSQSSPLREGILMAVDHLDDVDEILSQSLEVIPRHQSSSNGPAPDRSGSSASLSNVANVCVASTEGFESEEEILVRLREILDLNKQELINASIRRITFMFGFKDGSYPKYYTFNGPNYNENETIRHIEPALAFQLELGRLSNFNIKPIFTDNRNIHVYEAVSKTSPLDKRFFTRGIIRTGHIRDDISIQEYLTSEANRLMSDILDNLEVTDTSNSDLNHIFINFIAVFDISPEDVEAAFGGFLERFGKRLLRLRVSSAEIRIIIKDPQTGAPVPLRALINNVSGYVIKTEMYTEVKNAKGEWVFKSLGKPGSMHLRPIATPYPVKEWLQPKRYKAHLMGTTYVYDFPELFRQASSSQWKNFSADVKLTDDFFISNELIEDENGELTEVEREPGANAIGMVAFKITVKTPEYPRGRQFVVVANDITFKIGSFGPQEDEFFNKVTEYARKRGIPRIYLAANSGARIGMAEEIVPLFQVAWNDAANPDKGFQYLYLTSEGMETLKKFDKENSVLTERTVINGEERFVIKTIIGSEDGLGVECLRGSGLIAGATSRAYHDIFTITLVTCRSVGIGAYLVRLGQRAIQVEGQPIILTGAPAINKMLGREVYTSNLQLGGTQIMYNNGVSHLTAVDDLAGVEKIVEWMSYVPAKRNMPVPILETKDTWDRPVDFTPTNDETYDVRWMIEGRETESGFEYGLFDKGSFFETLSGWAKGVVVGRARLGGIPLGVIGVETRTVENLIPADPANPNSAETLIQEPGQVWHPNSAFKTAQAINDFNNGEQLPMMILANWRGFSGGQRDMFNEVLKYGSFIVDALVDYKQPIIIYIPPTGELRGGSWVVVDPTINADQMEMYADVNARAGVLEPQGMVGIKFRREKLLDTMNRLDDKYRELRSQLSNKSLAPEVHQQISKQLADRERELLPIYGQISLQFADLHDRSSRMVAKGVISKELEWTEARRFFFWRLRRRLNEEYLIKRLSHQVGEASRLEKIARIRSWYPASVDHEDDRQVATWIEENYKTLDDKLKGLKLESFAQDLAKKIRSDHDNAIDGLSEVIKMLSTDDKEKLLKTLK

SEQ ID NO: 24 - protein, 2233 aa, Saccharomyces cerevisiae
MSEESLFESSPQKMEYEITNYSERHTELPGHFIGLNTVDKLEESPLRDFVKSHGGHTVISKILIANNGIAAVKEIRSVRKWAYETFGDDRTVQFVAMATPEDLEANAEYIRMADQYIEVPGGTNNNNYANVDLIVDIAERADVDAVWAGWGHASENPLLPEKLSQSKRKVIFIGPPGNAMRSLGDKISSTIVAQSAKVPCIPWSGTGVDTVHVDEKTGLVSVDDDIYQKGCCTSPEDGLQKAKRIGFPVMIKASEGGGGKGIRQVEREEDFIALYHQAANEIPGSPIFIMKLAGRARHLEVQLLADQYGTNISLFGRDCSVQRRHQKIIEEAPVTIAKAETFHEMEKAAVRLGKLVGYVSAGTVEYLYSHDDGKFYFLELNPRLQVEHPTTEMVSGVNLPAAQLQIAMGIPMHRISDIRTLYGMNPHSASEIDFEFKTQDATKKQRRPIPKGHCTACRITSEDPNDGFKPSGGTLHELNFRSSSNVWGYFSVGNNGNIHSFSDSQFGHIFAFGENRQASRKHMVVALKELSIRGDFRTTVEYLIKLLETEDFEDNTITTGWLDDLITHKMTAEKPDPTLAVICGAATKAFLASEEARHKYIESLQKGQVLSKDLLQTMFPVDFIHEGKRYKFTVAKSGNDRYTLFINGSKCDIILRQLSDGGLLIAIGGKSHTIYWKEEVAATRLSVDSMTTLLEVENDPTQLRTPSPGKLVKFLVENGEHIIKGQPYAEIEVMKMQMPLVSQENGIVQLLKQPGSTIVAGDIMAIMTLDDPSKVKHALPFEGMLPDFGSPVIEGTKPAYKFKSLVSTLENILKGYDNQVIMNASLQQLIEVLRNPKLPYSEWKLHISALHSRLPAKLDEQMEELVARSLRRGAVFPARQLSKLIDMAVKNPEYNPDKLLGAVVEPLADIAHKYSNGLEAHEHSIFVHFLEEYYEVEKLFNGPNVREENIILKLRDENPKDLDKVALTVLSHSKVSAKNNLILAILKHYQPLCKLSSKVSAIFSTPLQHIVELESKATAKVALQAREILIQGALPSVKERTEQIEHILKSSVVKVAYGSSNPKRSEPDLNILKDLIDSNYVVFDVLLQFLTHQDPVVTAAAAQVYIRRAYRAYTIGDIRVHEGVTVPIVEWKFQLPSAAFSTFPTVKSKMGMNRAVPVSDLSYVANSQSSPLREGILMAVDHLDDVDEILSQSLEVIPRHQSSSNGPAPDRSGSSASLSNVANVCVASTEGFESEEEILVRLREILDLNKQELINASIRRITFMFGFKDGSYPKYYTFNGPNYNENETIRHIEPALAFQLELGRLSNFNIKPIFTDNRNIHVYEAVSKTSPLDKRFFTRGIIRTGHIRDDISIQEYLTSEANRLMSDILDNLEVTDTSNSDLNHIFINFIAVFDISPEDVEAAFGGFLERFGKRLLRLRVSSAEIRIIIKDPQTGAPVPLRALINNVSGYVIKTEMYTEVKNAKGEWVFKSLGKPGSMHLRPIATPYPVKEWLQPKRYKAHLMGTTYVYDFPELFRQASSSQWKNFSADVKLTDDFFISNELIEDENGELTEVEREPGANAIGMVAFKITVKTPEYPRGRQFVVVANDITFKIGSFGPQEDEFFNKVTEYARKRGIPRIYLAANSGARIGMAEEIVPLFQVAWNDAANPDKGFQYLYLTSEGMETLKKFDKENSVLTERTVINGEERFVIKTIIGSEDGLGVECLRGSGLIAGATSRAYHDIFTITLVTCRSVGIGAYLVRLGQRAIQVEGQPIILTGAPAINKMLGREVYTSNLQLGGTQIMYNNGVSHLTAVDDLAGVEKIVEWMSYVPAKRNMPVPILETKDTWDRPVDFTPTNDETYDVRWMIEGRETESGFEYGLFDKGSFFETLSGWAKGVVVGRARLGGIPLGVIGVETRTVENLIPADPANPNSAETLIQEPGQVWHPNSAFKTAQAINDFNNGEQLPMMILANWRGFSGGQRDMFNEVLKYGSFIVDALVDYKQPIIIYIPPTGELRGGSWVVVDPTINADQMEMYADVNARAGVLEPQGMVGIKFRREKLLDTMNRLDDKYRELRSQLSNKSLAPEVHQQISKQLADRERELLPIYGQISLQFADLHDRSSRMVAKGVISKELEWTEARRFFFWRLRRRLNEEYLIKRLSHQVGEASRLEKIARIRSWYPASVDHEDDRQVATWIEENYKTLDDKLKGLKLESFAQDLAKKIRSDHDNAIDGLSEVIKMLSTDDKEKLLKTLK

SEQ ID NO: 25 - protein, 2233 aa, Saccharomyces cerevisiae
MSEESLFESSPQKMEYEITNYSERHTELPGHFIGLNTVDKLEESPLRDFVKSHGGHTVISKILIANNGIAAVKEIRSVRKWAYETFGDDRTVQFVAMATPEDLEANAEYIRMADQYIEVPGGTNNNNYANVDLIVDIAERADVDAVWAGWGHASENPLLPEKLSQSKRKVIFIGPPGNAMRSLGDKISSTIVAQSAKVPCIPWSGTGVDTVHVDEKTGLVSVDDDIYQKGCCTSPEDGLQKAKRIGFPVMIKASEGGGGKGIRQVEREEDFIALYHQAANEIPGSPIFIMKLAGRARHLEVQLLADQYGTNISLFGRDCSVQRRHQKIIEEAPVTIAKAETFHEMEKAAVRLGKLVGYVSAGTVEYLYSHDDGKFYFLELNPRLQVEHPTTEMVSGVNLPAAQLQIAMGIPMHRISDIRTLYGMNPHSASEIDFEFKTQDATKKQRRPIPKGHCTACRITSEDPNDGFKPSGGTLHELNFRSSSNVWGYFSVGNNGNIHSFSDSQFGHIFAFGENRQASRKHMVVALKELSIRGDFRTTVEYLIKLLETEDFEDNTITTGWLDDLITHKMTAEKPDPTLAVICGAATKAFLASEEARHKYIESLQKGQVLSKDLLQTMFPVDFIHEGKRYKFTVAKSGNDRYTLFINGSKCDIILRQLPDGGLLIAIGGKSHTIYWKEEVAATRLSVDSMTTLLEVENDPTQLRTPSPGKLVKFLVENGEHIIKGQPYAEIEVMKMQMPLVSQENGIVQLLKQPGSTIVAGDIMAIMTLDDPSKVKHALPFEGMLPDFGSPVIEGTKPAYKFKSLVSTLENILKGYDNQVIMNASLQQLIEVLRNPKLPYSEWKLHISALHSRLPAKLDEQMEELVARSLRRGAVFPARQLSKLIDMAVKNPEYNPDKLLGAVVEPLADIAHKYSNGLEAHEHSIFVHFLEEYYEVEKLFNGPNVREENIILKLRDENPKDLDKVALTVLSHSKVSAKNNLILAILKHYQPLCKLSSKVSAIFSTPLQHIVELESKATAKVALQAREILIQGALPSVKERTEQIEHILKSSVVKVAYGSSNPKRSEPDLNILKDLIDSNYVVFDVLLQFLTHQDPVVTAAAAQVYIRRAYRAYTIGDIRVHEGVTVPIVEWKFQLPSAAFSTFPTVKSKMGMNRAVPVSDLSYVANSQSSPLREGILMAVDHLDDVDEILSQSLEVIPRHQSSSNGPAPDRSGSSASLSNVANVCVASTEGFESEEEILVRLREILDLNKQELINASIRRITFMFGFKDGSYPKYYTFNGPNYNENETIRHIEPALAFQLELGRLSNFNIKPIFTDNRNIHVYEAVSKTSPLDKRFFTRGIIRTGHIRDDISIQEYLTSEANRLMSDILDNLEVTDTSNSDLNHIFINFIAVFDISPEDVEAAFGGFLERFGKRLLRLRVSSAEIRIIIKDPQTGAPVPLRALINNVSGYVIKTEMYTEVKNAKGEWVFKSLGKPGSMHLRPIATPYPVKEWLQPKRYKAHLMGTTYVYDFPELFRQASSSQWKNFSADVKLTDDFFISNELIEDENGELTEVEREPGANAIGMVAFKITVKTPEYPRGRQFVVVANDITFKIGSFGPQEDEFFNKVTEYARKRGIPRIYLAANSGARIGMAEEIVPLFQVAWNDAANPDKGFQYLYLTSEGMETLKKFDKENSVLTERTVINGEERFVIKTIIGSEDGLGVECLRGSGLIAGATSRAYHDIFTITLVTCRSVGIGAYLVRLGQRAIQVEGQPIILTGAPAINKMLGREVYTSNLQLGGTQIMYNNGVSHLTAVDDLAGVEKIVEWMSYVPAKRNMPVPILETKDTWDRPVDFTPTNDETYDVRWMIEGRETESGFEYGLFDKGSFFETLSGWAKGVVVGRARLGGIPLGVIGVETRTVENLIPADPANPNSAETLIQEPGQVWHPNSAFKTAQAINDFNNGEQLPMMILANWRGFSGGQRDMFNEVLKYGSFIVDALVDYKQPIIIYIPPTGELRGGSWVVVDPTINADQMEMYADVNARAGVLEPQGMVGIKFRREKLLDTMNRLDDKYRELRSQLSNKSLAPEVHQQISKQLADRERELLPIYGQISLQFADLHDRSSRMVAKGVISKELEWTEARRFFFWRLRRRLNEEYLIKRLSHQVGEASRLEKIARIRSWYPASVDHEDDRQVATWIEENYKTLDDKLKGLKLESFAQDLAKKIRSDHDNAIDGLSEVIKMLSTDDKEKLLKTLK

SEQ ID NO: 26 - DNA, 420 bp, pTEF1 promoter
gcacacaccatagcttcaaaatgtttctactccttttttactcttccagattttctcggactccgcgcatcgccgtaccacttcaaaacacccaagcacagcatactaaatttcccctctttcttcctctagggtgtcgttaattacccgtactaaaggtttggaaaagaaaaaagagaccgcctcgtttctttttcttcgtcgaaaaaggcaataaaaatttttatcacgtttctttttcttgaaaatttttttttttgatttttttctctttcgatgacctcccattgatatttaagttaataaacggtcttcaatttctcaagtttcagtttcatttttcttgttctattacaactttttttacttcttgctcattagaaagaaagcatagcaatctaatctaagttttaattacaa